European Patent Application EP 4 599 667 A2, published August 13, 2025. Title: BREMIA LACTUCAE RESISTANT PLANTS. Applicant: Rijk Zwaan Zaadteelt en Zaadhandel B.V. Application EP. The sequence listing filed with the application follows.

SEQUENCE LISTING (11 sequences)

SEQ ID NO: 1 - DNA, 182 bp, Lactuca sativa
  misc_feature 1..182: note = source = /organism="Lactuca sativa" /mol_type="unassigned DNA"
  source 1..182: mol_type = genomic DNA
ttattctgctgccaacaagaacatggctgtgacctggggagagaatacactctatgactacttgctaaaccctaagaaggtacaagaccacatatatcatttgaaacttgagaggtcctaattcacatcacattttcttttttcttttttcttttttcttataaattgtgaaactcatgttg

SEQ ID NO: 2 - DNA, 175 bp, Lactuca sativa
  misc_feature 1..175: note = source = /organism="Lactuca sativa" /mol_type="unassigned DNA"
  source 1..175: mol_type = genomic DNA
ttattctgctgccaacaagaatatggctgtgacctggggagagaatacactctatgactacttactaaaccctaagaaggtacaagactacatatatcatttgaaacttgaaaggtcctaattcacatcacattttcttttttcttttttcttataaattgtgaaactcatgttg

SEQ ID NO: 3 - DNA, 195 bp, Lactuca sativa
  misc_feature 1..195: note = source = /organism="Lactuca sativa" /mol_type="unassigned DNA"
  source 1..195: mol_type = genomic DNA
tttttttttggtaaacagcatatctccagtctccttgatccttctttctctcctgcaaccataagacatgtatctgtttaagatttagccttggtttctaactttatgatcagtgccctttcaactttcttcttcaagtaagatgagttaccccttaatcctaactcaaattcccccaatattcttgttcaatta

SEQ ID NO: 4 - DNA, 189 bp, Lactuca sativa
  misc_feature 1..189: note = source = /organism="Lactuca sativa" /mol_type="unassigned DNA"
  source 1..189: mol_type = genomic DNA
tttttttttggtaaacagcatatctccttgatccttctttctctcctgcaaccataagacatgtatcggtttaagatttagccttggtttctaactttatgatcagtgccctttcaacttttcttctttaagtaagatgagttacccctaaatcctaattcaaattcccccaatattcttattcaatta

SEQ ID NO: 5 - DNA, 126 bp, Lactuca sativa
  misc_feature 1..126: note = source = /organism="Lactuca sativa" /mol_type="unassigned DNA"
  source 1..126: mol_type = genomic DNA
cttcttctacaacatgatttcggatacacttacggcagtccaccagtctccgcccaatacaccccgccgtcgaattgcccatcaaccgattttgcgaaaattgttctcgaatggacagctacatgt

SEQ ID NO: 6 - DNA, 20 bp, Lactuca sativa
  misc_feature 1..20: note = source = /organism="Lactuca sativa" /mol_type="unassigned DNA"
  source 1..20: mol_type = genomic DNA
ctttttggaaggcaatctgg

SEQ ID NO: 7 - DNA, 20 bp, Lactuca sativa
  misc_feature 1..20: note = source = /organism="Lactuca sativa" /mol_type="unassigned DNA"
  source 1..20: mol_type = genomic DNA
tccagggaaaaccatctttg

SEQ ID NO: 8 - DNA, 20 bp, Lactuca sativa
  misc_feature 1..20: note = source = /organism="Lactuca sativa" /mol_type="unassigned DNA"
  source 1..20: mol_type = genomic DNA
ccgtatgccgttcatcttct

SEQ ID NO: 9 - DNA, 20 bp, Lactuca sativa
  misc_feature 1..20: note = source = /organism="Lactuca sativa" /mol_type="unassigned DNA"
  source 1..20: mol_type = genomic DNA
gcactccaattgaatgatcg

SEQ ID NO: 10 - DNA, 20 bp, Lactuca sativa
  misc_feature 1..20: note = source = /organism="Lactuca sativa" /mol_type="unassigned DNA"
  source 1..20: mol_type = genomic DNA
acacaaaaccctgctcaacc

SEQ ID NO: 11 - DNA, 20 bp, Lactuca sativa
  misc_feature 1..20: note = source = /organism="Lactuca sativa" /mol_type="unassigned DNA"
  source 1..20: mol_type = genomic DNA
cgatcgaattgacgaccttt